European Patent Application EP 4 174 089 A1, published May 3, 2023. Title: ANTI-TIM3 SINGLE-CHAIN ANTIBODY AND USE THEREOF IN PREPARING MEDICINE FOR TREATING TUMOR. Applicant: Beijing Neurosurgical Institute. The sequence listing filed with the application follows.

SEQUENCE LISTING (6 sequences)

SEQ ID NO: 1 - protein, 232 aa, Artificial Sequence
  This sequence is synthesized in lab.
QVQLQQSGPGLVKPSHTLSLTCTVSGGSISSGGYYWSWTRQHPGMGLEWIGYISYSGSIYYTPSLKSRLTISVDTSKNQFSLKLSSVTAADTAVYYCASLDSWGSNRDYWGQGTLVTVSSGGGGSEIVLTQSPATLSLSPGERATLSCRASQSVSSYLAWYQQKPGQAPRLLIYDASNRATGIPARFSGSGSGTDFTLTISSLEPEDFAVYYCQQRSNWPLTFGGGTKVEIK

SEQ ID NO: 2 - DNA, 696 bp, Artificial Sequence
  This sequence is synthesized in lab.
caggtgcagctacagcagtcgggcccaggactggtgaagccttcacacaccctgtccctcacctgcactgtctctggtggctccatcagcagtggtggttactactggagttggacccgtcagcacccagggatgggcctggagtggattggatacatctcttacagtgggagtatctattacactccgtccctcaagagtcgacttaccatatcagtggacacgtctaagaaccagttctccctgaagctgagctctgtgactgccgcggacacggccgtatattactgtgcgagtttggattcctggggatctaaccgtgactactggggccagggaaccctggtcaccgtctcgagtggaggtggtggatccgaaattgtgttgacgcagtctccagccaccctgtctttgtctccaggggaaagagccaccctctcctgcagggccagtcagagtgttagcagctacttagcctggtaccaacagaaacctggccaggctcccaggctcctcatctatgatgcatccaacagggccactggcatcccagccaggttcagtggcagtgggtctgggacagacttcactctcaccatcagcagcctagagcctgaagattttgcagtttattactgtcagcagcgtagcaactggccgctcactttcggcggagggaccaaggtggagattaag

SEQ ID NO: 3 - protein, 998 aa, Artificial Sequence
  This sequence is synthesized in lab.
QVQLVESGGGVVQPGRSLRLSCAASGFTFSSYGMHWVRQAPGKGLEWVAVIWYDGSNKFYADSVKGRFTISRDNSKNTLYLQMNSLRAEDTAVYYCARRSDYRGYYGMDVWGQGTTVTVSSGSTSGGGSGGGSGGGGSSEIVLTQSPATLSLSPGERATLSCRASQSVINYLAWYQQKPGQAPRLLIYDASNRASGIPARFSGSGSGTDFTLTISSLEPEDFAVYYCQQRRNWPLTFGGGTKVEIKGGGGSGGGGSGGGGSQVQLVQSGAEVKKPGASVKVSCKASGYTFTDFEMHWVRQAPGQGLEWMGDIDPGTGDTAYNLKFKGRVTMTTDTSTSTAYMELRSLRSDDTAVYYCALGAFVYWGQGTLVTVSSGSTSGGGSGGGSGGGGSSDVVMTQSPLSLPVTPGEPASISCRSSQSLANSYGNTYLSWYLQKPGQSPQLLIYGISNRFSGVPDRFSGSGSGTDFTLKISRVEAEDVGVYYCLQGTHQPYTFGQGTKLEIKTTTPAPRPPTPAPTIASQPLSLRPEACRPAAGGAVHTRGLDFACDIYIWAPLAGTCGVLLLSLVITLYCRSKRSRLLHSDYMNMTPRRPGPTRKHYQPYAPPRDFAAYRSRVKFSRSADAPAYKQGQNQLYNELNLGRREEYDVLDKRRGRDPEMGGKPRRKNPQEGLYNELQKDKMAEAYSEIGMKGERRRGKGHDGLYQGLSTATKDTYDALHMQALPPREGRGSLLTCGDVEENPGPMTNKCLLQIALLLCFSTTALSQVQLQQSGPGLVKPSHTLSLTCTVSGGSISSGGYYWSWTRQHPGMGLEWIGYISYSGSIYYTPSLKSRLTISVDTSKNQFSLKLSSVTAADTAVYYCASLDSWGSNRDYWGQGTLVTVSSGGGGSEIVLTQSPATLSLSPGERATLSCRASQSVSSYLAWYQQKPGQAPRLLIYDASNRATGIPARFSGSGSGTDFTLTISSLEPEDFAVYYCQQRSNWPLTFGGGTKVEIK

SEQ ID NO: 4 - DNA, 2994 bp, Artificial Sequence
  This sequence is synthesized in lab.
caggtgcagctggtggagtctgggggaggcgtggtccagcctgggaggtccctgagactctcctgtgcagcgtctggattcaccttcagtagctatggcatgcactgggtccgccaggctccaggcaaggggctggagtgggtggcagttatatggtatgatggaagtaataaattctatgcagactccgtgaagggccgattcaccatctccagagacaattccaagaacacgctgtatctgcaaatgaacagcctgagagccgaggacacggctgtgtattactgtgcgaggagaagtgactacaggggctactacggtatggacgtctggggccaagggaccacggtcaccgtctcctcaggcagtactagcggtggtggctccgggggcggttccggtgggggcggcagcagcgaaattgtgttgacacagtctccagccaccctgtctttgtctccaggggaaagagccaccctctcctgcagggccagtcagagtgttatcaactacttagcctggtaccaacagaaacctggccaggctcccaggctcctcatctatgatgcatccaacagggcctctggcatcccagccaggttcagtggcagtgggtctgggacagacttcactctcaccatcagcagcctagagcctgaagattttgcagtttattactgtcagcagcgtcgcaactggccgctcactttcggcggagggaccaaggtggagatcaaaggaggtggtggatccggaggtggtggctccggaggtggtggatcccaggttcagctggtgcagtctggagctgaggtgaagaagcctggggcctcagtgaaggtctcctgcaaggcttctggttacacctttaccgactttgaaatgcactgggtgcgacaggcccctggacaagggcttgagtggatgggagatattgatcctggaactggtgatactgcctacaatctgaagttcaagggcagagtcaccatgaccacagacacatccacgagcacagcctacatggagctgaggagcctgaggtctgacgacacggccgtgtattactgtgcgttgggggcctttgtttactggggccagggaaccctggtcaccgtctcctcaggcagtactagcggtggtggctccgggggcggttccggtgggggcggcagcagcgatgttgtgatgactcagtctccactctccctgcccgtcacccctggagagccggcctccatctcctgcaggtctagtcagagtcttgcaaacagttatgggaacacctatttgtcttggtacctgcagaagccagggcagtctccacagctcctgatctatgggatttccaacagattttctggggtccctgacaggttcagtggcagtggatcaggcacagattttacactgaaaatcagcagagtggaggctgaggacgttggggtttattactgcttacaaggtacacatcagccgtacacgtttggccaggggaccaagctggagatcaaaaccactaccccagcaccgaggccacccaccccggctcctaccatcgcctcccagcctctgtccctgcgtccggaggcatgtagacccgcagctggtggggccgtgcatacccggggtcttgacttcgcctgcgatatctacatttgggcccctctggctggtacttgcggggtcctgctgctttcactcgtgatcactctttactgtaggagtaagaggagcaggctcctgcacagtgactacatgaacatgactccccgccgccccgggcccacccgcaagcattaccagccctatgccccaccacgcgacttcgcagcctatcgctcccgcgtgaaattcagccgcagcgcagatgctccagcctacaagcaggggcagaaccagctctacaacgaactcaatcttggtcggagagaggagtacgacgtgctggacaagcggagaggacgggacccagaaatgggcgggaagccgcgcagaaagaatccccaagagggcctgtacaacgagctccaaaaggataagatggcagaagcctatagcgagattggtatgaaaggggaacgcagaagaggcaaaggccacgacggactgtaccagggactcagcaccgccaccaaggacacctatgacgctcttcacatgcaggccctgccgcctcgggagggaaggggttctctcctgacctgcggcgatgtggaggagaaccccggacccatgaccaacaagtgtctcctccaaattgctctcctgttgtgcttctccactacagctctttcccaggtgcagctacagcagtcgggcccaggactggtgaagccttcacacaccctgtccctcacctgcactgtctctggtggctccatcagcagtggtggttactactggagttggacccgtcagcacccagggatgggcctggagtggattggatacatctcttacagtgggagtatctattacactccgtccctcaagagtcgacttaccatatcagtggacacgtctaagaaccagttctccctgaagctgagctctgtgactgccgcggacacggccgtatattactgtgcgagtttggattcctggggatctaaccgtgactactggggccagggaaccctggtcaccgtctcgagtggaggtggtggatccgaaattgtgttgacgcagtctccagccaccctgtctttgtctccaggggaaagagccaccctctcctgcagggccagtcagagtgttagcagctacttagcctggtaccaacagaaacctggccaggctcccaggctcctcatctatgatgcatccaacagggccactggcatcccagccaggttcagtggcagtgggtctgggacagacttcactctcaccatcagcagcctagagcctgaagattttgcagtttattactgtcagcagcgtagcaactggccgctcactttcggcggagggaccaaggtggagattaag

SEQ ID NO: 5 - DNA, 2181 bp, Artificial Sequence
  This sequence is synthesized in lab.
caggtgcagctggtggagtctgggggaggcgtggtccagcctgggaggtccctgagactctcctgtgcagcgtctggattcaccttcagtagctatggcatgcactgggtccgccaggctccaggcaaggggctggagtgggtggcagttatatggtatgatggaagtaataaattctatgcagactccgtgaagggccgattcaccatctccagagacaattccaagaacacgctgtatctgcaaatgaacagcctgagagccgaggacacggctgtgtattactgtgcgaggagaagtgactacaggggctactacggtatggacgtctggggccaagggaccacggtcaccgtctcctcaggcagtactagcggtggtggctccgggggcggttccggtgggggcggcagcagcgaaattgtgttgacacagtctccagccaccctgtctttgtctccaggggaaagagccaccctctcctgcagggccagtcagagtgttatcaactacttagcctggtaccaacagaaacctggccaggctcccaggctcctcatctatgatgcatccaacagggcctctggcatcccagccaggttcagtggcagtgggtctgggacagacttcactctcaccatcagcagcctagagcctgaagattttgcagtttattactgtcagcagcgtcgcaactggccgctcactttcggcggagggaccaaggtggagatcaaaggaggtggtggatccggaggtggtggctccggaggtggtggatcccaggttcagctggtgcagtctggagctgaggtgaagaagcctggggcctcagtgaaggtctcctgcaaggcttctggttacacctttaccgactttgaaatgcactgggtgcgacaggcccctggacaagggcttgagtggatgggagatattgatcctggaactggtgatactgcctacaatctgaagttcaagggcagagtcaccatgaccacagacacatccacgagcacagcctacatggagctgaggagcctgaggtctgacgacacggccgtgtattactgtgcgttgggggcctttgtttactggggccagggaaccctggtcaccgtctcctcaggcagtactagcggtggtggctccgggggcggttccggtgggggcggcagcagcgatgttgtgatgactcagtctccactctccctgcccgtcacccctggagagccggcctccatctcctgcaggtctagtcagagtcttgcaaacagttatgggaacacctatttgtcttggtacctgcagaagccagggcagtctccacagctcctgatctatgggatttccaacagattttctggggtccctgacaggttcagtggcagtggatcaggcacagattttacactgaaaatcagcagagtggaggctgaggacgttggggtttattactgcttacaaggtacacatcagccgtacacgtttggccaggggaccaagctggagatcaaaaccactaccccagcaccgaggccacccaccccggctcctaccatcgcctcccagcctctgtccctgcgtccggaggcatgtagacccgcagctggtggggccgtgcatacccggggtcttgacttcgcctgcgatatctacatttgggcccctctggctggtacttgcggggtcctgctgctttcactcgtgatcactctttactgtaggagtaagaggagcaggctcctgcacagtgactacatgaacatgactccccgccgccccgggcccacccgcaagcattaccagccctatgccccaccacgcgacttcgcagcctatcgctcccgcgtgaaattcagccgcagcgcagatgctccagcctacaagcaggggcagaaccagctctacaacgaactcaatcttggtcggagagaggagtacgacgtgctggacaagcggagaggacgggacccagaaatgggcgggaagccgcgcagaaagaatccccaagagggcctgtacaacgagctccaaaaggataagatggcagaagcctatagcgagattggtatgaaaggggaacgcagaagaggcaaaggccacgacggactgtaccagggactcagcaccgccaccaaggacacctatgacgctcttcacatgcaggccctgccgcctcgg

SEQ ID NO: 6 - protein, 727 aa, Artificial Sequence
  This sequence is synthesized in lab.
QVQLVESGGGVVQPGRSLRLSCAASGFTFSSYGMHWVRQAPGKGLEWVAVIWYDGSNKFYADSVKGRFTISRDNSKNTLYLQMNSLRAEDTAVYYCARRSDYRGYYGMDVWGQGTTVTVSSGSTSGGGSGGGSGGGGSSEIVLTQSPATLSLSPGERATLSCRASQSVINYLAWYQQKPGQAPRLLIYDASNRASGIPARFSGSGSGTDFTLTISSLEPEDFAVYYCQQRRNWPLTFGGGTKVEIKGGGGSGGGGSGGGGSQVQLVQSGAEVKKPGASVKVSCKASGYTFTDFEMHWVRQAPGQGLEWMGDIDPGTGDTAYNLKFKGRVTMTTDTSTSTAYMELRSLRSDDTAVYYCALGAFVYWGQGTLVTVSSGSTSGGGSGGGSGGGGSSDVVMTQSPLSLPVTPGEPASISCRSSQSLANSYGNTYLSWYLQKPGQSPQLLIYGISNRFSGVPDRFSGSGSGTDFTLKISRVEAEDVGVYYCLQGTHQPYTFGQGTKLEIKTTTPAPRPPTPAPTIASQPLSLRPEACRPAAGGAVHTRGLDFACDIYIWAPLAGTCGVLLLSLVITLYCRSKRSRLLHSDYMNMTPRRPGPTRKHYQPYAPPRDFAAYRSRVKFSRSADAPAYKQGQNQLYNELNLGRREEYDVLDKRRGRDPEMGGKPRRKNPQEGLYNELQKDKMAEAYSEIGMKGERRRGKGHDGLYQGLSTATKDTYDALHMQALPPR